European Patent Application EP 4 279 128 A2, published November 22, 2023. Title: NOVEL ANTIBODY BINDING TO TFPI AND COMPOSITION COMPRISING THE SAME. Applicant: MOGAM INSTITUTE FOR BIOMEDICAL RESEARCH. Application EP, filed December 29, 2015. The sequence listing filed with the application follows.

SEQUENCE LISTING (203 sequences)

SEQ ID NO: 1 - protein, 118 aa, synthetic construct
  REGION 1..118: note = Clone T417_mouse Variable heavy chain
EVHLVESGGDLVKPGGSLKLSCAASGFTFSSYAMSWVRQTPDKRLEWVATITTGGSYTYYPDSVKGRFTISRDNAKNTLYLQMSSLKSEDTAMYYCARQDGNFLMDYWGQGTTVTVSS

SEQ ID NO: 2 - protein, 113 aa, synthetic construct
  REGION 1..113: note = Clone T417_mouse Variable light chain
DVVMTQTPLTLSVTIGQPASISCKSSQSLLDSDGKTYLNWLLQRPGQSPKRLIYLVSKLDSGVPDRFTGSGSGTDFTLKISRVEAEDLGVYYCWQGTHFPFTFGSGTKLEIKR

SEQ ID NO: 3 - protein, 120 aa, synthetic construct
  REGION 1..120: note = Clone T308_mouse Variable heavy chain
EVKLVESGGGLVKPGGSLKLSCAASGFTFSNYPMSWVRQTPEKRLEWVATISNSGSYTYYPDSVKGRFTISRDNAKNTLYLQMNSLRSEDTAMYYCARQVYGNYEDFDYWGQGTTLTVSS

SEQ ID NO: 4 - protein, 113 aa, synthetic construct
  REGION 1..113: note = Clone T308_mouse Variable light chain
DVVMTQTPLTLSVTIGQPASISCKSSQSLLDSDGKTYLNWLLQRPGQSPKRLIYLVSKLDSGVPDRFTGSGSGTDFTLKISRVEAEDLGVYYCWQGTHFPYTFGGGTKLELKR

SEQ ID NO: 5 - protein, 5 aa, synthetic construct
  REGION 1..5: note = Clone T417_mouse Variable heavy chain CDR 1
SYAMS

SEQ ID NO: 6 - protein, 17 aa, synthetic construct
  REGION 1..17: note = Clone T417_mouse Variable heavy chain CDR 2
TITTGGSYTYYPDSVKG

SEQ ID NO: 7 - protein, 9 aa, synthetic construct
  REGION 1..9: note = Clone T417_mouse Variable heavy chain CDR 3
QDGNFLMDY

SEQ ID NO: 8 - protein, 16 aa, synthetic construct
  REGION 1..16: note = Clone T417_mouse Variable light chain CDR 1
KSSQSLLDSDGKTYLN

SEQ ID NO: 9 - protein, 7 aa, synthetic construct
  REGION 1..7: note = Clone T417_mouse Variable light chain CDR 2
LVSKLDS

SEQ ID NO: 10 - protein, 8 aa, synthetic construct
  REGION 1..8: note = Clone T417_mouse Variable light chain CDR 3
WQGTHFPF

SEQ ID NO: 11 - protein, 5 aa, synthetic construct
  REGION 1..5: note = Clone T308_mouse Variable heavy chain CDR 1
NYPMS

SEQ ID NO: 12 - protein, 17 aa, synthetic construct
  REGION 1..17: note = Clone T308_mouse Variable heavy chain CDR 2
TISNSGSYTYYPDSVKG

SEQ ID NO: 13 - protein, 11 aa, synthetic construct
  REGION 1..11: note = Clone T308_mouse Variable heavy chain CDR 3
QVYGNYEDFDY

SEQ ID NO: 14 - protein, 16 aa, synthetic construct
  REGION 1..16: note = Clone T308_mouse Variable light chain CDR 1
KSSQSLLDSDGKTYLN

SEQ ID NO: 15 - protein, 7 aa, synthetic construct
  REGION 1..7: note = Clone T308_mouse Variable light chain CDR 2
LVSKLDS

SEQ ID NO: 16 - protein, 8 aa, synthetic construct
  REGION 1..8: note = Clone T308_mouse Variable light chain CDR 3
WQGTHFPY

SEQ ID NO: 17 - DNA, 87 bp, synthetic construct
  misc_feature 1..87: note = Primer_T417VH-F
  source 1..87: mol_type = other DNA
gcggccgccatgtatctgggtctgaactatgtctttatcgtgtttctgctgaatggtgtgcagtctgaggtgcacctggtggagtct

SEQ ID NO: 18 - DNA, 43 bp, synthetic construct
  misc_feature 1..43: note = Primer_T417VH Apa-R
  source 1..43: mol_type = other DNA
nnnngggccccttggtgctggctgaggagacggtgaccgtggt

SEQ ID NO: 19 - DNA, 95 bp, synthetic construct
  misc_feature 1..95: note = Primer_T417 VL-F
  source 1..95: mol_type = other DNA
gcggccgccatggatagccaggctcaggtgctgatgctgctgctgctgtgggtgtcagggacttgcggggacgttgtgatgacccagactccact

SEQ ID NO: 20 - DNA, 31 bp, synthetic construct
  misc_feature 1..31: note = Primer_VL-R
  source 1..31: mol_type = other DNA
nnnnggtaccagatttcaactgctcatcaga

SEQ ID NO: 21 - protein, 118 aa, synthetic construct
  REGION 1..118: note = Clone 308_humanized Variable heavy chain
EVQLVESGGGLVKPGGSLRLSCAASGFTFSSYAMNWVRQAPGKGLEWVSTITTGGSYTYYADSVKGRFTISRDNAKNSLYLQMNSLRAEDTAVYYCARQDGNFLMDYWGQGTLVTVSS

SEQ ID NO: 22 - protein, 113 aa, synthetic construct
  REGION 1..113: note = Clone 308_humanized Variable light chain
DVVMTQTPLSLPVTLGQPASISCKSSQSLLDSDGKTYLNWLQQRPGQSPKRLIYLVSKLDSGVPDRFTGSGSGTDFTLKISRVEAEDVGVYYCWQGTHFPFTFGQGTKVEIKR

SEQ ID NO: 23 - protein, 5 aa, synthetic construct
  REGION 1..5: note = Clone 308_humanized Variable heavy chain CDR 1
SYAMN

SEQ ID NO: 24 - protein, 118 aa, synthetic construct
  REGION 1..118: note = Clone 308-2_humanized and mutated Variable heavy chain
EVQLVESGGGLVKPGGSLRLSCAASGFTFSSYAMNWVRQAPGKGLEWVSTITTGGSYTYYADSVQGRFTISRDNAKNSLYLQMNSLRAEDTAVYYCARQDGNFLMDYWGQGTLVTVSS

SEQ ID NO: 25 - protein, 118 aa, synthetic construct
  REGION 1..118: note = Clone 308-4_humanized and mutated Variable heavy chain
EVQLVESGGGLVKPGGSLRLSCAASGFTFSSYAMNWVRQAPGKGLEWVSTITTGGSYTYYADSVEGRFTISRDNAKNSLYLQMNSLRAEDTAVYYCARQDGNFLMDYWGQGTLVTVSS

SEQ ID NO: 26 - protein, 17 aa, synthetic construct
  REGION 1..17: note = Clone 308-2_humanized and mutated Variable heavy chain CDR 2
TITTGGSYTYYPDSVQG

SEQ ID NO: 27 - protein, 17 aa, synthetic construct
  REGION 1..17: note = Clone 308-4_humanized and mutated Variable heavy chain CDR 2
TITTGGSYTYYPDSVEG

SEQ ID NO: 28 - DNA, 50 bp, synthetic construct
  misc_feature 1..50: note = Primer_VH Fo
  source 1..50: mol_type = other DNA
tgctgtgggtgagtggtacctgtggggaagtgcagctcgtggagagcggt

SEQ ID NO: 29 - DNA, 56 bp, synthetic construct
  misc_feature 1..56: note = Primer_VH Re
  source 1..56: mol_type = other DNA
agtgggaacacggagggccccttggtgctggcggatgagacagtcacaagtgtccc

SEQ ID NO: 30 - protein, 58 aa, synthetic construct
  REGION 1..58: note = Human_TFPI Kunitz domain 2
KPDFCFLEEDPGICRGYITRYFYNNQTKQCERFKYGGCLGNMNNFETLEECKNICEDG

SEQ ID NO: 31 - protein, 58 aa, synthetic construct
  REGION 1..58: note = Rabbit_TFPI Kunitz domain 2
KPDFCFLEEDPGICRGFMTRYFYNNQSKQCEQFKYGGCLGNSNNFETLEECRNTCEDP

SEQ ID NO: 32 - protein, 58 aa, synthetic construct
  REGION 1..58: note = Mouse_TFPI Kunitz domain 2
RPDFCFLEEDPGLCRGYMKRYLYNNQTKQCERFVYGGCLGNRNNFETLDECKKICENP

SEQ ID NO: 33 - DNA, 29 bp, synthetic construct
  misc_feature 1..29: note = Primer_HTK2 For
  source 1..29: mol_type = other DNA
ccatggaaacccgacttttgcttcctgga

SEQ ID NO: 34 - DNA, 30 bp, synthetic construct
  misc_feature 1..30: note = Primer_RTK2 For
  source 1..30: mol_type = other DNA
ccatggaaacccgatttctgctttctggag

SEQ ID NO: 35 - DNA, 30 bp, synthetic construct
  misc_feature 1..30: note = Primer_MTK2 For
  source 1..30: mol_type = other DNA
ccatggagacctgacttctgctttctggag

SEQ ID NO: 36 - DNA, 33 bp, synthetic construct
  misc_feature 1..33: note = Primer_HTK2 Re
  source 1..33: mol_type = other DNA
gcggccgcctagccgtcttcacagatgttcttg

SEQ ID NO: 37 - DNA, 30 bp, synthetic construct
  misc_feature 1..30: note = Primer_RTK2 Re
  source 1..30: mol_type = other DNA
gcggccgcctaggggtcctcacaggtgttg

SEQ ID NO: 38 - DNA, 37 bp, synthetic construct
  misc_feature 1..37: note = Primer_MTK2 Re
  source 1..37: mol_type = other DNA
gcggccgcctaggggttctcacagattttcttgcatt

SEQ ID NO: 39 - protein, 304 aa, synthetic construct
  REGION 1..304: note = HUMAN Tissue factor pathway inhibitor
MIYTMKKVHALWASVCLLLNLAPAPLNADSEEDEEHTIITDTELPPLKLMHSFCAFKADDGPCKAIMKRFFFNIFTRQCEEFIYGGCEGNQNRFESLEECKKMCTRDNANRIIKTTLQQEKPDFCFLEEDPGICRGYITRYFYNNQTKQCERFKYGGCLGNMNNFETLEECKNICEDGPNGFQVDNYGTQLNAVNNSLTPQSTKVPSLFEFHGPSWCLTPADRGLCRANENRFYYNSVIGKCRPFKYSGCGGNENNFTSKQECLRACKKGFIQRISKGGLIKTKRKRKKQRVKIAYEEIFVKNM

SEQ ID NO: 40 - DNA, 27 bp, synthetic construct
  misc_feature 1..27: note = VH FR1 Fo
  source 1..27: mol_type = other DNA
gaagtccagctggtggagtctggaggt

SEQ ID NO: 41 - DNA, 57 bp, synthetic construct
  misc_feature 1..57: note = VH FR1 Re_S
  source 1..57: mol_type = other DNA
cggggcctgacgaacccagttcatggcatagctgctgaaggtgaagccgctcgctgc

SEQ ID NO: 42 - DNA, 57 bp, synthetic construct
  misc_feature 1..57: note = VH FR1 Re_H
  source 1..57: mol_type = other DNA
cggggcctgacgaacccagttcatggcataatggctgaaggtgaagccgctcgctgc

SEQ ID NO: 43 - DNA, 57 bp, synthetic construct
  misc_feature 1..57: note = VH FR1 Re_K
  source 1..57: mol_type = other DNA
cggggcctgacgaacccagttcatggcatatttgctgaaggtgaagccgctcgctgc

SEQ ID NO: 44 - DNA, 57 bp, synthetic construct
  misc_feature 1..57: note = VH FR1 Re_R
  source 1..57: mol_type = other DNA
cggggcctgacgaacccagttcatggcatatctgctgaaggtgaagccgctcgctgc

SEQ ID NO: 45 - DNA, 57 bp, synthetic construct
  misc_feature 1..57: note = VH FR1 Re_T
  source 1..57: mol_type = other DNA
cggggcctgacgaacccagttcatggcataagtgctgaaggtgaagccgctcgctgc

SEQ ID NO: 46 - DNA, 57 bp, synthetic construct
  misc_feature 1..57: note = VH FR1 Re_Y
  source 1..57: mol_type = other DNA
cggggcctgacgaacccagttcatggcataatagctgaaggtgaagccgctcgctgc

SEQ ID NO: 47 - DNA, 57 bp, synthetic construct
  misc_feature 1..57: note = VH FR1 Re_I
  source 1..57: mol_type = other DNA
cggggcctgacgaacccagttcatggcataaatgctgaaggtgaagccgctcgctgc

SEQ ID NO: 48 - DNA, 57 bp, synthetic construct
  misc_feature 1..57: note = VH FR1 Re_L
  source 1..57: mol_type = other DNA
cggggcctgacgaacccagttcatggcataaaggctgaaggtgaagccgctcgctgc

SEQ ID NO: 49 - DNA, 27 bp, synthetic construct
  misc_feature 1..27: note = VH FR2 Fo
  source 1..27: mol_type = other DNA
tatgccatgaactgggttcgtcaggcc

SEQ ID NO: 50 - DNA, 93 bp, synthetic construct
  misc_feature 1..93: note = VH FR2 Re_T-YH-EQDH
  source 1..93: mol_type = other DNA
gttatcgcgggaaatggtgaagcgcccttgaacgctatcggcgtagtaggtgtttgacccaccggttgtgatggtgctgacccattccaagcc

SEQ ID NO: 51 - DNA, 93 bp, synthetic construct
  misc_feature 1..93: note = VH FR2 Re_T-RK-EQDH
  source 1..93: mol_type = other DNA
gttatcgcgggaaatggtgaagcgcccttgaacgctatcggcgtagtaggttyttgacccaccggttgtgatggtgctgacccattccaagcc

SEQ ID NO: 52 - DNA, 93 bp, synthetic construct
  misc_feature 1..93: note = VH FR2 Re_FYLH-YH-EQDH
  source 1..93: mol_type = other DNA
gttatcgcgggaaatggtgaagcgcccttgaacgctatcggcgtagtaggtgtttgacccacctwrtgtgatggtgctgacccattccaagcc

SEQ ID NO: 53 - DNA, 93 bp, synthetic construct
  misc_feature 1..93: note = VH FR2 Re_FYLH-RK-EQDH
  source 1..93: mol_type = other DNA
gttatcgcgggaaatggtgaagcgcccttgaacgctatcggcgtagtaggttyttgacccacctwrtgtgatggtgctgacccattccaagcc

SEQ ID NO: 54 - DNA, 93 bp, synthetic construct
  misc_feature 1..93: note = VH FR2 Re_KRI-YH-EQDH
  source 1..93: mol_type = other DNA
gttatcgcgggaaatggtgaagcgcccttgaacgctatcggcgtagtaggtgtttgacccaccthttgtgatggtgctgacccattccaagcc

SEQ ID NO: 55 - DNA, 93 bp, synthetic construct
  misc_feature 1..93: note = VH FR2 Re_KRI-RK-EQDH
  source 1..93: mol_type = other DNA
gttatcgcgggaaatggtgaagcgcccttgaacgctatcggcgtagtaggttyttgacccaccthttgtgatggtgctgacccattccaagcc

SEQ ID NO: 56 - DNA, 93 bp, synthetic construct
  misc_feature 1..93: note = VH FR2 Re_T-YH-EQDH_#2
  source 1..93: mol_type = other DNA
gttatcgcgggaaatggtgaagcgcccntsaacgctatcggcgtagtaggtatrtgacccaccggttgtgatggtgctgacccattccaagcc

SEQ ID NO: 57 - DNA, 93 bp, synthetic construct
  misc_feature 1..93: note = VH FR2 Re_T-RK-EQDH_#2
  source 1..93: mol_type = other DNA
gttatcgcgggaaatggtgaagcgcccntsaacgctatcggcgtagtaggttyttgacccaccggttgtgatggtgctgacccattccaagcc

SEQ ID NO: 58 - DNA, 93 bp, synthetic construct
  misc_feature 1..93: note = VH FR2 Re_FYLH-YH-EQDH_#2
  source 1..93: mol_type = other DNA
gttatcgcgggaaatggtgaagcgcccntsaacgctatcggcgtagtaggtatrtgacccacctwrtgtgatggtgctgacccattccaagcc

SEQ ID NO: 59 - DNA, 93 bp, synthetic construct
  misc_feature 1..93: note = VH FR2 Re_FYLH-RK-EQDH_#2
  source 1..93: mol_type = other DNA
gttatcgcgggaaatggtgaagcgcccntsaacgctatcggcgtagtaggttyttgacccacctwrtgtgatggtgctgacccattccaagcc

SEQ ID NO: 60 - DNA, 93 bp, synthetic construct
  misc_feature 1..93: note = VH FR2 Re_KRI-YH-EQDH_#2
  source 1..93: mol_type = other DNA
gttatcgcgggaaatggtgaagcgcccntsaacgctatcggcgtagtaggtatrtgacccaccthttgtgatggtgctgacccattccaagcc

SEQ ID NO: 61 - DNA, 93 bp, synthetic construct
  misc_feature 1..93: note = VH FR2 Re_KRI-RK-EQDH_#2
  source 1..93: mol_type = other DNA
gttatcgcgggaaatggtgaagcgcccntsaacgctatcggcgtagtaggttyttgacccaccthttgtgatggtgctgacccattccaagcc

SEQ ID NO: 62 - DNA, 27 bp, synthetic construct
  misc_feature 1..27: note = VH FR3 Fo
  source 1..27: mol_type = other DNA
gggcgcttcaccatttcccgcgataac

SEQ ID NO: 63 - DNA, 60 bp, synthetic construct
  misc_feature 1..60: note = VH FR3 Re_N
  source 1..60: mol_type = other DNA
gccctggccccaataatccatcagaaaattgccatcctggcgcgcgcaataatataccgc

SEQ ID NO: 64 - DNA, 60 bp, synthetic construct
  misc_feature 1..60: note = VH FR3 Re_F
  source 1..60: mol_type = other DNA
gccctggccccaataatccatcagaaaaaagccatcctggcgcgcgcaataatataccgc

SEQ ID NO: 65 - DNA, 60 bp, synthetic construct
  misc_feature 1..60: note = VH FR3 Re_H
  source 1..60: mol_type = other DNA
gccctggccccaataatccatcagaaaatggccatcctggcgcgcgcaataatataccgc

SEQ ID NO: 66 - DNA, 60 bp, synthetic construct
  misc_feature 1..60: note = VH FR3 Re_K
  source 1..60: mol_type = other DNA
gccctggccccaataatccatcagaaatttgccatcctggcgcgcgcaataatataccgc

SEQ ID NO: 67 - DNA, 60 bp, synthetic construct
  misc_feature 1..60: note = VH FR3 Re_Q
  source 1..60: mol_type = other DNA
gccctggccccaataatccatcagaaattggccatcctggcgcgcgcaataatataccgc

SEQ ID NO: 68 - DNA, 60 bp, synthetic construct
  misc_feature 1..60: note = VH FR3 Re_R
  source 1..60: mol_type = other DNA
gccctggccccaataatccatcagaaatctgccatcctggcgcgcgcaataatataccgc

SEQ ID NO: 69 - DNA, 60 bp, synthetic construct
  misc_feature 1..60: note = VH FR3 Re_Y
  source 1..60: mol_type = other DNA
gccctggccccaataatccatcagaaaatagccatcctggcgcgcgcaataatataccgc

SEQ ID NO: 70 - DNA, 54 bp, synthetic construct
  misc_feature 1..54: note = VH Final Fo
  source 1..54: mol_type = other DNA
ggttctggtggtggtggttctgctagcgacgtggtgatgacacagacgccgctg

SEQ ID NO: 71 - DNA, 48 bp, synthetic construct
  misc_feature 1..48: note = VH Final Re
  source 1..48: mol_type = other DNA
ggagctcacagtcaccagcgtgccctggccccaataatccatcagaaa

SEQ ID NO: 72 - DNA, 27 bp, synthetic construct
  misc_feature 1..27: note = VL FR1 Fo
  source 1..27: mol_type = other DNA
gacgtggtgatgacacagacgccgctg

SEQ ID NO: 73 - DNA, 57 bp, synthetic construct
  misc_feature 1..57: note = VL FR1 Re_S
  source 1..57: mol_type = other DNA
gagccaattcagatacgtcttgccgtcggagtccagcagcgactggcttgatttgca

SEQ ID NO: 74 - DNA, 57 bp, synthetic construct
  misc_feature 1..57: note = VL FR1 Re_I
  source 1..57: mol_type = other DNA
gagccaattcagatacgtcttgccgtcaatgtccagcagcgactggcttgatttgca

SEQ ID NO: 75 - DNA, 57 bp, synthetic construct
  misc_feature 1..57: note = VL FR1 Re_L
  source 1..57: mol_type = other DNA
gagccaattcagatacgtcttgccgtcaaggtccagcagcgactggcttgatttgca

SEQ ID NO: 76 - DNA, 57 bp, synthetic construct
  misc_feature 1..57: note = VL FR1 Re_N
  source 1..57: mol_type = other DNA
gagccaattcagatacgtcttgccgtcagcgtccagcagcgactggcttgatttgca

SEQ ID NO: 77 - DNA, 57 bp, synthetic construct
  misc_feature 1..57: note = VL FR1 Re_Q
  source 1..57: mol_type = other DNA
gagccaattcagatacgtcttgccgtcttggtccagcagcgactggcttgatttgca

SEQ ID NO: 78 - DNA, 57 bp, synthetic construct
  misc_feature 1..57: note = VL FR1 Re_R
  source 1..57: mol_type = other DNA
gagccaattcagatacgtcttgccgtctctgtccagcagcgactggcttgatttgca

SEQ ID NO: 79 - DNA, 57 bp, synthetic construct
  misc_feature 1..57: note = VL FR1 Re_F
  source 1..57: mol_type = other DNA
gagccaattcagatacgtcttgccgtcaaagtccagcagcgactggcttgatttgca

SEQ ID NO: 80 - DNA, 57 bp, synthetic construct
  misc_feature 1..57: note = VL FR1 Re_K
  source 1..57: mol_type = other DNA
gagccaattcagatacgtcttgccgtctttgtccagcagcgactggcttgatttgca

SEQ ID NO: 81 - DNA, 57 bp, synthetic construct
  misc_feature 1..57: note = VL FR1 Re_T
  source 1..57: mol_type = other DNA
gagccaattcagatacgtcttgccgtcagtgtccagcagcgactggcttgatttgca

SEQ ID NO: 82 - DNA, 57 bp, synthetic construct
  misc_feature 1..57: note = VL FR1 Re_V
  source 1..57: mol_type = other DNA
gagccaattcagatacgtcttgccgtcaacgtccagcagcgactggcttgatttgca

SEQ ID NO: 83 - DNA, 30 bp, synthetic construct
  misc_feature 1..30: note = VL FR2 Fo
  source 1..30: mol_type = other DNA
gacggcaagacgtatctgaattggctccag

SEQ ID NO: 84 - DNA, 75 bp, synthetic construct
  misc_feature 1..75: note = VL FR2 Re_T-YH
  source 1..75: mol_type = other DNA
gcgtttaatttcaaccttagtgccttggccgaacgtaaacggaaagtrggtgccctgccagcaatagtagacgcc

SEQ ID NO: 85 - DNA, 75 bp, synthetic construct
  misc_feature 1..75: note = VL FR2 Re_T-LIHQNK
  source 1..75: mol_type = other DNA
gcgtttaatttcaaccttagtgccttggccgaacgtaaacggaaawwkggtgccctgccagcaatagtagacgcc

SEQ ID NO: 86 - DNA, 75 bp, synthetic construct
  misc_feature 1..75: note = VL FR2 Re_FYIN-YH
  source 1..75: mol_type = other DNA
gcgtttaatttcaaccttagtgccttggccgaacgtaaacggaaagtrawwgccctgccagcaatagtagacgcc

SEQ ID NO: 87 - DNA, 75 bp, synthetic construct
  misc_feature 1..75: note = VL FR2 Re_FYIN-LIHQNK
  source 1..75: mol_type = other DNA
gcgtttaatttcaaccttagtgccttggccgaacgtaaacggaaawwkawwgccctgccagcaatagtagacgcc

SEQ ID NO: 88 - DNA, 39 bp, synthetic construct
  misc_feature 1..39: note = VL Final Re
  source 1..39: mol_type = other DNA
gcgtttaatttcaaccttagtgccttggccgaacgtaaa

SEQ ID NO: 89 - DNA, 43 bp, synthetic construct
  misc_feature 1..43: note = VL Final Fo SfiI
  source 1..43: mol_type = other DNA
cgtggcccaggcggccgacgtggtgatgacacagacgccgctg

SEQ ID NO: 90 - DNA, 33 bp, synthetic construct
  misc_feature 1..33: note = VL Final Fo NruI
  source 1..33: mol_type = other DNA
ctatcgcgattgcagtggcactggctggtttcg

SEQ ID NO: 91 - DNA, 96 bp, synthetic construct
  misc_feature 1..96: note = VL Overlapping Fo
  source 1..96: mol_type = other DNA
ggcacgctggtgactgtgagctccggaggcggcggaagtggcggaggaggcagcggcggaggcgggagtgacgtggtgatgacacagacgccgctg

SEQ ID NO: 92 - DNA, 72 bp, synthetic construct
  misc_feature 1..72: note = VL Final Re
  source 1..72: mol_type = other DNA
gtcctcttcagaaataagcttttgttcggatccgcgtttaatttcaaccttagtgccttggccgaacgtaaa

SEQ ID NO: 93 - DNA, 66 bp, synthetic construct
  misc_feature 1..66: note = VH Homologous recombination
  source 1..66: mol_type = other DNA
gctctgcaggctagtggtggtggtggttctggtggtggtggttctggtggtggtggttctgctagc

SEQ ID NO: 94 - DNA, 60 bp, synthetic construct
  misc_feature 1..60: note = VL Homologous recombination
  source 1..60: mol_type = other DNA
ttgttatcagatctcgagctattacaagtcctcttcagaaataagcttttgttcggatcc

SEQ ID NO: 95 - protein, 118 aa, synthetic construct
  REGION 1..118: note = Clone 1001_Variable heavy chain
EVQLVESGGGLVKPGGSLRLSCAASGFTFSSYAMNWVRQAPGKGLEWVSTITTGGSYTYYADSVDGRFTISRDNAKNSLYLQMNSLRAEDTAVYYCARQDGNFLMDYWGQGTLVTVSS

SEQ ID NO: 96 - protein, 113 aa, synthetic construct
  REGION 1..113: note = Clone 1001_Variable light chain
DVVMTQTPLSLPVTLGQPASISCKSSQSLLDIDGKTYLNWLQQRPGQSPKRLIYLVSKLDSGVPDRFTGSGSGTDFTLKISRVEAEDVGVYYCWQGTHFPFTFGQGTKVEIKR

SEQ ID NO: 97 - protein, 118 aa, synthetic construct
  REGION 1..118: note = Clone 1015_Variable heavy chain
EVQLVESGGGLVKPGGSLRLSCAASGFTFSSYAMNWVRQAPGKGLEWVSTITTGGSHTYYADSVEGRFTISRDNAKNSLYLQMNSLRAEDTAVYYCARQDGNFLMDYWGQGTLVTVSS

SEQ ID NO: 98 - protein, 118 aa, synthetic construct
  REGION 1..118: note = Clone 1021_Variable heavy chain
EVQLVESGGGLVKPGGSLRLSCAASGFTFSSYAMNWVRQAPGKGLEWVSTITTGGSYTYYADSVDGRFTISRDNAKNSLYLQMNSLRAEDTAVYYCARQDGHFLMDYWGQGTLVTVSS

SEQ ID NO: 99 - protein, 118 aa, synthetic construct
  REGION 1..118: note = Clone 1023_Variable heavy chain
EVQLVESGGGLVKPGGSLRLSCAASGFTFSSYAMNWVRQAPGKGLEWVGTITTGGSYTYYADSVDGRFTISRDNAKNSLYLQMNSLRAEDTAVYYCARQDGNFLMDYWGQGTLVTVSS

SEQ ID NO: 100 - protein, 118 aa, synthetic construct
  REGION 1..118: note = Clone 1024_Variable heavy chain
EVQLVESGGGLVKPGGSLRLSCAASGFTFSSYAMSWVRQAPGKGLEWVSTITTGGSYTYYADSVDGRFTISRDNAKNSLYLQMNSLRAEDTAVYYCARQDGNFLMDYWGQGTLVTVSS

SEQ ID NO: 101 - protein, 113 aa, synthetic construct
  REGION 1..113: note = Clone 1024_Variable light chain
DVVMTQTPLSLPVTLGQPASISCKSSQSLLDLDGKTYLNWLQQRPGQSPKRLIYLVSKLDSGVPDRFTGSGSGTDFTLKISRVEAEDVGVYYCWQGTHFPFTFGQGTKVEIKR

SEQ ID NO: 102 - protein, 118 aa, synthetic construct
  REGION 1..118: note = Clone 1104_Variable heavy chain
EVQLVESGGGLVKPGGSLRLSCAASGFTFSSYAMNWVRQAPGKGLEWVGTITTGGSHTYYADSVQGRFTISRDNAKNSLYLQMNSLRAEDTAVYYCARQDGNFLMDYWGQGTLVTVSS

SEQ ID NO: 103 - protein, 113 aa, synthetic construct
  REGION 1..113: note = Clone 1104_Variable light chain
DVVMTQTPLSLPVTLGQPASISCKSSQSLLDVDGKTYLNWLQQRPGQSPKRLIYLVSKLDSGVPDRFTGSGSGTDFTLKISRVEAEDVGVYYCWQGTHFPFTFGQGTKVEIKR

SEQ ID NO: 104 - protein, 118 aa, synthetic construct
  REGION 1..118: note = Clone 1123_Variable heavy chain
EVQLVESGGGLVKPGGSLRLSCAASGFTFSSYAMNWVRQAPGKGLEWVSTITTGGSHTYYADSVEGRFTISRDNAKNSLYLQMNSLRAEDTAVYYCARQDGHFLMDYWGQGTLVTVSS

SEQ ID NO: 105 - protein, 118 aa, synthetic construct
  REGION 1..118: note = Clone 1202_Variable heavy chain
EVQLVESGGGLVKPGGSLRLSCAASGFTFSSYAMNWVRQAPGKGLEWVGTITTGGSYTYYADSVDGRFTISRDNAKNSLYLKMNSLRAEDTAVYYCARQDGNFLMDYWGQGTLVTVSS

SEQ ID NO: 106 - protein, 113 aa, synthetic construct
  REGION 1..113: note = Clone 1208_Variable light chain
DVVMTQTPLSLPVTLGQPASISCKSSQSLLDVDGKTYLNWLQQRPGQSPKRLIYLVSKLDSGVPDRFTGSGSGTDFTLKISRVEAEDVGVYYCWQGTYLPFTFGQGTKVEIKR

SEQ ID NO: 107 - protein, 118 aa, synthetic construct
  REGION 1..118: note = Clone 1216_Variable heavy chain
EVQLVESGGGLVKPGGSLRLSCAASGFTFSHYAMNWVRQAPGKGLEWVSTITTGGSYTYYADSVEGRFTISRDNAKNSLYLQMNSLRAEDTAVYYCARQDGHFLMDYWGQGTLVTVSS

SEQ ID NO: 108 - protein, 113 aa, synthetic construct
  REGION 1..113: note = Clone 1216_Variable light chain
DVVMTQTPLSLPVTLGQPASISCKSSQSLLDIDGKTYLNWLQQRPGQSPKRLIYLVSKLDSGVPDRFTGSGSGTDFTLKISRVEAEDVGVYYCWQGTHLPFTFGQGTKVEIKR

SEQ ID NO: 109 - protein, 118 aa, synthetic construct
  REGION 1..118: note = Clone 1223_Variable heavy chain
EVQLVESGGGLVKPGGSLRLSCAASGFTFSSYAMNWVRQAPGKGLEWVSTITTGGSYTYYADSVEGRFTISRDNAKNSLYLQMNSLRAEDTAVYYCARQDGHFLMDYWGQGTLVTVSS

SEQ ID NO: 110 - protein, 118 aa, synthetic construct; identical to SEQ ID NO: 24
  REGION 1..118: note = Clone 1234_Variable heavy chain

SEQ ID NO: 111 - protein, 113 aa, synthetic construct
  REGION 1..113: note = Clone 1234_Variable light chain
DVVMTQTPLSLPVTLGQPASISCKSSQSLLDIDGKTYLNWLQQRPGQSPKRLIYLVSKLDSGVPDRFTGSGSGTDFTLEISRVEAEDVGVYYCWQGTHFPFTFGQGTKVEIKR

SEQ ID NO: 112 - protein, 118 aa, synthetic construct
  REGION 1..118: note = Clone 1243_Variable heavy chain
EVQLVESGGGLVKPGGSLRLSCAASGFTFSSYAMNWVRQAPGKGLEWVSTITTGGSHTYYADSVHGRFTISRDNAKNSLYLQMNSLRAEDTAVYYCARQDGHFLMDYWGQGTLVTVSS

SEQ ID NO: 113 - protein, 118 aa, synthetic construct
  REGION 1..118: note = Clone 1248_Variable heavy chain
EVQLVESGGGLVKPGGSLRLSCAASGFTFSSYAMNWVRQAPGKGLEWVSTITTGGSHTYYADSVDGRFTISRDNAKNSLYLQMNSLRAEDTAVYYCARQDGHFLMDYWGQGTLVTVSS

SEQ ID NO: 114 - protein, 118 aa, synthetic construct
  REGION 1..118: note = Clone 3007_Variable heavy chain
EVQLVESGGGLVKPGGSLRLSCAASGFTFTSYAMNWVRQAPGKGLEWVSTITLGGSYTYYADSVQGRFTISRDNAKNSLYLQMNSLRAEDTAVYYCARQDGNFLMDYWGQGTLVTVSS

SEQ ID NO: 115 - protein, 118 aa, synthetic construct; identical to SEQ ID NO: 97
  REGION 1..118: note = Clone 3016_Variable heavy chain

SEQ ID NO: 116 - protein, 113 aa, synthetic construct
  REGION 1..113: note = Clone 3016_Variable light chain
DVVMTQTPLSLPVTLGQPASISCKSSQSLLDSDGKTYLNWLQQRPGQSPKRLIYLVSKLDSGVPDRFTGSGSGTDFTLKISRVEAEDVGVYYCWQGTHLPFTFGQGTKVEIKR

SEQ ID NO: 117 - protein, 118 aa, synthetic construct
  REGION 1..118: note = Clone 3024_Variable heavy chain
EVQLVESGGGLVKPGGSLRLSCAASGFTFSSYAMSWVRQAPGKGLEWVSTITTGGSYTYYADSVQGRFTISRDNAKNSLYLQMNSLRAEDTAVYYCARQDGNFLMDYWGQGTLVTVSS

SEQ ID NO: 118 - protein, 118 aa, synthetic construct
  REGION 1..118: note = Clone 3120_Variable heavy chain
EVQLVESGGGLVKPGGSLRLSCAASGFTFSSYAMNWVRQAPGKGLEWVSTITTGGSYTYYADSVEGRFTISRDNAKNSLYLQMNSLRAEDTAVYYCARQDGYFLMDYWGQGTLVTVSS

SEQ ID NO: 119 - protein, 118 aa, synthetic construct
  REGION 1..118: note = Clone 3131_Variable heavy chain
EVQLVESGGGLVKPGGSLRLSCAASGFTFSSYAMSWVRQAPGKGLEWVSTITTGGSYTYYADSVQGRFTISRDNAKNSLYLQMNSLRAEDTAVYYCARQDGQFLMDYWGQGTLVTVSS

SEQ ID NO: 120 - protein, 118 aa, synthetic construct
  REGION 1..118: note = Clone 3203_Variable heavy chain
EVQLVESGGGLVKPGGSLRLSCAASGFTFSSYAMSWVRQAPGKGLEWVSTITTGGSYTYYADSVEGRFTISRDNAKNSLYLQMNSLRAEDTAVYYCARQDGNFLMDYWGQGTLVTVSS

SEQ ID NO: 121 - protein, 118 aa, synthetic construct
  REGION 1..118: note = Clone 4011_Variable heavy chain
EVQLVESGGGLVKPGGSLRLSCAASGFTFYSYAMNWVRQAPGKGLEWVSTITTGGSHTYYADSVEGRFTISRDNAKNSLYLQMNSLRAEDTAVYYCARQDGNFLMDYWGQGTLVTVSS

SEQ ID NO: 122 - protein, 113 aa, synthetic construct
  REGION 1..113: note = Clone 4011_Variable light chain
DVVMTQTPLSLPVTLGQPASISCKSSQSLLDVDGKTYLNWLQQRPGQSPKRLIYLVSKLDSGVPDRFTGSGSGTDFTLKISRVEAEDVGVYYCWQGTHLPFTFGQGTKVEIKR

SEQ ID NO: 123 - protein, 118 aa, synthetic construct
  REGION 1..118: note = Clone 4017_Variable heavy chain
EVQLVESGGGLVKPGGSLRLSCAASGFTFSSYAMNWVRQAPGKGLEWVGTITTGGSYTYYADSVQGRFTISRDNAKNSLYLQMNSLRAEDTAVYYCARQDGYFLMDYWGQGTLVTVSS

SEQ ID NO: 124 - protein, 118 aa, synthetic construct
  REGION 1..118: note = Clone 4034_Variable heavy chain
EVQLVESGGGLVKPGGSLRLSCAASGFTFSSYAMNWVRQAPGKGLEWVSTITTGGSHTYYADSVEGRFTISRDNAKNSLYLQMNSLRAEDTAVYYCARQDGYFLMDYWGQGTLVTVSS

SEQ ID NO: 125 - protein, 118 aa, synthetic construct
  REGION 1..118: note = Clone 4041_Variable heavy chain
EVQLVESGGGLVKPGGSLRLSCAASGFTFSSYAMSWVRQAPGKGLEWVSTITTGGSHTYYADSVEGRFTISRDNAKNSLYLQMNSLRAEDTAVYYCARQDGYFLMDYWGQGTLVTVSS

SEQ ID NO: 126 - protein, 118 aa, synthetic construct
  REGION 1..118: note = Clone 4141_Variable heavy chain
EVQLVESGGGLVKPGGSLRLSCAASGFTFSSYAMNWVRQAPGKGLEWVGTITTGGSHTYYADSVEGRFTISRDNAKNSLYLQMNSLRAEDTAVYYCARQDGYFLMDYWGQGTLVTVSS

SEQ ID NO: 127 - protein, 118 aa, synthetic construct; identical to SEQ ID NO: 118
  REGION 1..118: note = Clone 4146_Variable heavy chain

SEQ ID NO: 128 - protein, 118 aa, synthetic construct
  REGION 1..118: note = Clone 4206_Variable heavy chain
EVQLVESGGGLVKPGGSLRLSCAASGFTFSSYAMNWVRQAPGKGLEWVSTITTGGSHTYYADSVEGRFTISRDNAKNSLYLQMDSLRAEDTAVYYCARQDGNFLMDYWGQGTLVTVSS

SEQ ID NO: 129 - protein, 118 aa, synthetic construct
  REGION 1..118: note = Clone 4208_Variable heavy chain
EVQLVESGGGLVKSGGSLRLSCAASGFTFSSYAMSWVRQAPGKGLEWVGTITTGGSYTYYADSVQGRFTISRDNAKNSLYLQMNSLRAEDTAVYYCARQDGNFLMDYWGQGTLVTVSS

SEQ ID NO: 130 - protein, 113 aa, synthetic construct
  REGION 1..113: note = Clone 4208_Variable light chain
DVVMTQTPLSLPVTLGQPASISCKSSQSLLDTDGKTYLNWLQQRPGQSPKRLIYLVSKLDSGVPDRFTGSGSGTDFTLKISRVEAEDVGVYYCWQGTHFPFTFGQGTKVEIKR

SEQ ID NO: 131 - protein, 120 aa, synthetic construct
  REGION 1..120: note = Clone 4278_Variable heavy chain
EVQLVESGGGLVKPGGSLRLSCAASGFTFSKYAMNWFRQAPGKGLEWVSTITLGGSYTYYADSVDGRFTISRDNAKNSLYLQMNSLRAEDTAVYYCARQYLDGNFLMDYWGQGTLVTVSS

SEQ ID NO: 132 - protein, 120 aa, synthetic construct
  REGION 1..120: note = Clone 4287_Variable heavy chain
EVQLVESGGGLVKPGGSLRLSCAASGFTFSKYAMNWFRQAPGKGLEWVSTITTGGSYTYYADSVEGRFTISRDNAKNSLYLQMNSLRAEDTAVYYCARQHPYGNFLMDYWGQGTLVTVSS

SEQ ID NO: 133 - protein, 118 aa, synthetic construct
  REGION 1..118: note = Clone 4_Variable heavy chain
EVQLVESGGGLVKPGGSLRLSCAASGFTFSSYAMNWVRQAPGKGLEWVGTITTGGSHTYYADSVEGRFTISRDNAKNSLYLQMNSLRAEDTAVYYCARQDGNFLMDYWGQGTLVTVSS

SEQ ID NO: 134 - protein, 118 aa, synthetic construct
  REGION 1..118: note = Clone 6_Variable heavy chain
EVQLVESGGGLVKPGGSLRLSCAASGFTFSSYAMNWVRQAPGKGLEWVGTITTGGSYTYYADSVEGRFTISRDNAKNSLYLQMNSLRAEDTAVYYCARQDGNFLMDYWGQGTLVTVSS

SEQ ID NO: 135 - protein, 118 aa, synthetic construct
  REGION 1..118: note = Clone 9_Variable heavy chain
EVQLVESGGGLVKPGGSLRLSCAASGFTFSSYAMNWVRQAPGKGLEWVGTITTGGSYTYYADSVQGRFTISRDNAKNSLYLQMNSLRAEDTAVYYCARQDGNFLMDYWGQGTLVTVSS

SEQ ID NO: 136 - protein, 118 aa, synthetic construct; identical to SEQ ID NO: 134
  REGION 1..118: note = Clone 11_Variable heavy chain

SEQ ID NO: 137 - protein, 118 aa, synthetic construct
  REGION 1..118: note = Clone 12_Variable heavy chain
EVQLVESGGGLVKPGGSLRLSCAASGFTFSSYAMNWVRQAPGKGLEWVGTITTGGSHTYYADSVEGRFTISRDNAKNSLYLQMNSLRAEDTAVYYCARQDGHFLMDYWGQGTLVTVSS

SEQ ID NO: 138 - protein, 118 aa, synthetic construct; identical to SEQ ID NO: 133
  REGION 1..118: note = Clone 13_Variable heavy chain

SEQ ID NO: 139 - protein, 113 aa, synthetic construct
  REGION 1..113: note = Clone 14_Variable light chain
DVVMTQTPLSLPVTLGQPASISCKSSPSLLDSDGKTYLNWLQQRPGQSPKRLIYLVSKLDSGVPDRFTGSGSGTDFTLKISRVEAEDVGVYYCWQGTYFPFTFGQGTKVEIKR

SEQ ID NO: 140 - protein, 113 aa, synthetic construct
  REGION 1..113: note = Clone 15_Variable light chain
DVVMTQTPLSLPVTLGQPASISCKSSPSLLDSDGKTYLNWLQQRPGQSPKRLIYLVSKLDSGVPDRFTGSGSGTDFTLKISRVEAEDVGVYYCWQGFYFPFTFGQGTKVEIKR

SEQ ID NO: 141 - protein, 118 aa, synthetic construct
  REGION 1..118: note = Clone 16_Variable heavy chain
EVQLVESGGGLVKPGGSLRLSCAASGFTFSHYAMTWVRQAPGKGLEWVSTITTGGSHTYYADSVEGRFTISRDNAKNSLYLQMNSLRAEDTAVYYCARQDGNFLMDYWGQGTLVTVSS

SEQ ID NO: 142 - protein, 118 aa, synthetic construct
  REGION 1..118: note = Clone 17_Variable heavy chain
EVQLVESGGGLVKPGGSLRLSCAASGFTFSSYAMTWVRQAPGKGLEWVSTITTGGSHTYYADSVQGRFTISRDNAKNSLYLQMNSLRAEDTAVYYCARQDGNFLMDYWGQGTLVTVSS

SEQ ID NO: 143 - protein, 118 aa, synthetic construct
  REGION 1..118: note = Clone 18_Variable heavy chain
EVQLVESGGGLVKPGGSLRLSCAASGFTFSHYAMTWVRQAPGKGLEWVSTITTGGSHTYYADSVDGRFTISRDNAKNSLYLQMNSLRAEDTAVYYCARQDGNFLMDYWGQGTLVTVSS

SEQ ID NO: 144 - protein, 118 aa, synthetic construct
  REGION 1..118: note = Clone 19_Variable heavy chain
EVQLVESGGGLVKPGGSLRLSCAASGFTFSQYAMNWVRQAPGKGLEWVSTITKKGSFTYYADSVDGRFTISRDNAKNSLYLQMNSLRAEDTAVYYCARQDGEFLMDYWGQGTLVTVSS

SEQ ID NO: 145 - protein, 118 aa, synthetic construct
  REGION 1..118: note = Clone 20_Variable heavy chain
EVQLVESGGGLVKPGGSLRLSCAASGFTFSQYAMNWVRQAPGKGLEWVSTIKKGGSFTYYADSVDGRFTISRDNAKNSLYLQMNSLRAEDTAVYYCARQDGEFLMDYWGQGTLVTVSS

SEQ ID NO: 146 - protein, 118 aa, synthetic construct
  REGION 1..118: note = Clone 21_Variable heavy chain
EVQLVESGGGLVKPGGSLRLSCAASGFTFSSYAMNWVRQAPGKGLEWVSTITKGGSYTYYADSVDGRFTISRDNAKNSLYLQMNSLRAEDTAVYYCARQDGNFLMDYWGQGTLVTVSS

SEQ ID NO: 147 - protein, 113 aa, synthetic construct
  REGION 1..113: note = Clone 22_Variable light chain
DVVMTQTPLSLPVTLGQPASISCKSSPSLLDVDGKTYLNWLQQRPGQSPKRLIYLVSKLDSGVPDRFTGSGSGTDFTLKISRVEAEDVGVYYCWQGTYFPFTFGQGTKVEIKR

SEQ ID NO: 148 - protein, 118 aa, synthetic construct; identical to SEQ ID NO: 107
  REGION 1..118: note = Clone 23_Variable heavy chain

SEQ ID NO: 149 - protein, 5 aa, synthetic construct
  REGION 1..5: note = Clone 1001_Variable heavy chain CDR 1
SYAMN

SEQ ID NO: 150 - protein, 17 aa, synthetic construct
  REGION 1..17: note = Clone 1001_Variable heavy chain CDR 2
TITTGGSYTYYADSVDG

SEQ ID NO: 151 - protein, 9 aa, synthetic construct
  REGION 1..9: note = Clone 1001_Variable heavy chain CDR 3
QDGNFLMDY

SEQ ID NO: 152 - protein, 16 aa, synthetic construct
  REGION 1..16: note = Clone 1001_Variable light chain CDR 1
KSSQSLLDIDGKTYLN

SEQ ID NO: 153 - protein, 7 aa, synthetic construct
  REGION 1..7: note = Clone 1001_Variable light chain CDR 2
LVSKLDS

SEQ ID NO: 154 - protein, 8 aa, synthetic construct
  REGION 1..8: note = Clone 1001_Variable light chain CDR 3
WQGTHFPF

SEQ ID NO: 155 - protein, 17 aa, synthetic construct
  REGION 1..17: note = Clone 1015_Variable heavy chain CDR 2
TITTGGSHTYYADSVEG

SEQ ID NO: 156 - protein, 9 aa, synthetic construct
  REGION 1..9: note = Clone 1021_Variable heavy chain CDR 3
QDGHFLMDY

SEQ ID NO: 157 - protein, 5 aa, synthetic construct
  REGION 1..5: note = Clone 1024_Variable heavy chain CDR 1
SYAMS

SEQ ID NO: 158 - protein, 16 aa, synthetic construct
  REGION 1..16: note = Clone 1024_Variable light chain CDR 1
KSSQSLLDLDGKTYLN

SEQ ID NO: 159 - protein, 17 aa, synthetic construct
  REGION 1..17: note = Clone 1104_Variable heavy chain CDR 2
TITTGGSHTYYADSVQG

SEQ ID NO: 160 - protein, 16 aa, synthetic construct
  REGION 1..16: note = Clone 1104_Variable light chain CDR 1
KSSQSLLDVDGKTYLN

SEQ ID NO: 161 - protein, 8 aa, synthetic construct
  REGION 1..8: note = Clone 1208_Variable light chain CDR 3
WQGTYLPF

SEQ ID NO: 162 - protein, 17 aa, synthetic construct
  REGION 1..17: note = Clone 1214_Variable heavy chain CDR 2
TITTGGSYTYYADSVEG

SEQ ID NO: 163 - protein, 5 aa, synthetic construct
  REGION 1..5: note = Clone 1216_Variable heavy chain CDR 1
HYAMN

SEQ ID NO: 164 - protein, 8 aa, synthetic construct
  REGION 1..8: note = Clone 1216_Variable light chain CDR 3
WQGTHLPF

SEQ ID NO: 165 - protein, 17 aa, synthetic construct
  REGION 1..17: note = Clone 1234_Variable heavy chain CDR 2
TITTGGSYTYYADSVQG

SEQ ID NO: 166 - protein, 17 aa, synthetic construct
  REGION 1..17: note = Clone 1243_Variable heavy chain CDR 2
TITTGGSHTYYADSVHG

SEQ ID NO: 167 - protein, 17 aa, synthetic construct
  REGION 1..17: note = Clone 1248_Variable heavy chain CDR 2
TITTGGSHTYYADSVDG

SEQ ID NO: 168 - protein, 17 aa, synthetic construct
  REGION 1..17: note = Clone 3007_Variable heavy chain CDR 2
TITLGGSYTYYADSVQG

SEQ ID NO: 169 - protein, 16 aa, synthetic construct
  REGION 1..16: note = Clone 3016_Variable light chain CDR 1
KSSQSLLDSDGKTYLN

SEQ ID NO: 170 - protein, 9 aa, synthetic construct
  REGION 1..9: note = Clone 3120_Variable heavy chain CDR 3
QDGYFLMDY

SEQ ID NO: 171 - protein, 9 aa, synthetic construct
  REGION 1..9: note = Clone 3131_Variable heavy chain CDR 3
QDGQFLMDY

SEQ ID NO: 172 - protein, 5 aa, synthetic construct
  REGION 1..5: note = Clone 4278_Variable heavy chain CDR 1
KYAMN

SEQ ID NO: 173 - protein, 17 aa, synthetic construct
  REGION 1..17: note = Clone 4278_Variable heavy chain CDR 2
TITLGGSYTYYADSVDG

SEQ ID NO: 174 - protein, 11 aa, synthetic construct
  REGION 1..11: note = Clone 4278_Variable heavy chain CDR 3
QYLDGNFLMDY

SEQ ID NO: 175 - protein, 11 aa, synthetic construct
  REGION 1..11: note = Clone 4287_Variable heavy chain CDR 3
QHPYGNFLMDY

SEQ ID NO: 176 - protein, 16 aa, synthetic construct
  REGION 1..16: note = Clone 1_Variable light chain CDR 1
KSSPSLLDSDGKTYLN

SEQ ID NO: 177 - protein, 16 aa, synthetic construct
  REGION 1..16: note = Clone 2_Variable light chain CDR 1
KSSPSLLDIDGKTYLN

SEQ ID NO: 178 - protein, 16 aa, synthetic construct
  REGION 1..16: note = Clone 3_Variable light chain CDR 1
KSSPSLLDVDGKTYLN

SEQ ID NO: 179 - protein, 8 aa, synthetic construct
  REGION 1..8: note = Clone 14_Variable light chain CDR 3
WQGTYFPF

SEQ ID NO: 180 - protein, 8 aa, synthetic construct
  REGION 1..8: note = Clone 15_Variable light chain CDR 3
WQGFYFPF

SEQ ID NO: 181 - protein, 5 aa, synthetic construct
  REGION 1..5: note = Clone 16_Variable heavy chain CDR 1
HYAMT

SEQ ID NO: 182 - protein, 5 aa, synthetic construct
  REGION 1..5: note = Clone 17_Variable heavy chain CDR 1
SYAMT

SEQ ID NO: 183 - protein, 5 aa, synthetic construct
  REGION 1..5: note = Clone 19_Variable heavy chain CDR 1
QYAMN

SEQ ID NO: 184 - protein, 17 aa, synthetic construct
  REGION 1..17: note = Clone 19_Variable heavy chain CDR 2
TITKKGSFTYYADSVDG

SEQ ID NO: 185 - protein, 9 aa, synthetic construct
  REGION 1..9: note = Clone 19_Variable heavy chain CDR 3
QDGEFLMDY

SEQ ID NO: 186 - protein, 17 aa, synthetic construct
  REGION 1..17: note = Clone 20_Variable heavy chain CDR 2
TIKKGGSFTYYADSVDG

SEQ ID NO: 187 - protein, 17 aa, synthetic construct
  REGION 1..17: note = Clone 21_Variable heavy chain CDR 2
TITKGGSYTYYADSVDG

SEQ ID NO: 188 - protein, 5 aa, synthetic construct
  REGION 1..5: note = Clone 23_Variable heavy chain CDR 1
HYAMN

SEQ ID NO: 189 - DNA, 53 bp, synthetic construct
  misc_feature 1..53: note = VH Fo
  source 1..53: mol_type = other DNA
tgctgtgggtgagtggtacctgtggggaagtccagctggtggagtctggaggt

SEQ ID NO: 190 - DNA, 56 bp, synthetic construct
  misc_feature 1..56: note = VH Re
  source 1..56: mol_type = other DNA
agtgggaacacggagggccccttggtgctggcggagctcacagtcaccagcgtgcc

SEQ ID NO: 191 - DNA, 53 bp, synthetic construct
  misc_feature 1..53: note = VL Fo
  source 1..53: mol_type = other DNA
tgctgtgggtgagtggtacctgtggggacgtggtgatgacacagacgccgctg

SEQ ID NO: 192 - DNA, 66 bp, synthetic construct
  misc_feature 1..66: note = VL Re_CL overlap
  source 1..66: mol_type = other DNA
gatgaacacagaaggggcagccaccgtgcgtttaatttcaaccttagtgccttggccgaacgtaaa

SEQ ID NO: 193 - DNA, 27 bp, synthetic construct
  misc_feature 1..27: note = Ck Fo
  source 1..27: mol_type = other DNA
acggtggctgccccttctgtgttcatc

SEQ ID NO: 194 - DNA, 45 bp, synthetic construct
  misc_feature 1..45: note = Ck Re
  source 1..45: mol_type = other DNA
gattggatccaagcttactagcactcacccctgttgaaagactta

SEQ ID NO: 195 - protein, 118 aa, synthetic construct
  REGION 1..118: note = Clone A24_Variable heavy chain
EVQLVESGGGLVKPGGSLRLSCAASGFTFHSYAMNWVRQAPGKGLEWVSTITTRGSYTYYADSVEGRFTISRDNAKNSLYLQMNSLRAEDTAVYYCARQDGNFLMDYWGQGTLVTVSS

SEQ ID NO: 196 - protein, 113 aa, synthetic construct
  REGION 1..113: note = Clone A25_Variable light chain
DVVMTQTPLSLPVTLGQPASISCKSSQSLLDRDGKTYLNWLQQRPGQSPKRLIYLVSKLDSGVPDRFTGSGSGTDFTLKISRVEAEDVGVYYCWQGTHFPFTFGQGTKVEIKR

SEQ ID NO: 197 - protein, 118 aa, synthetic construct
  REGION 1..118: note = Clone A52_Variable heavy chain
EVQLVESGGGLVKPGGSLRLSCAASGFTFSSYAMNWVRQAPGKGLEWVSTITTGGSHTYYADSVDGRFTISRDNAKNSLYLQMNSLRAEDTAVYYCARQDGNFLMDYWGQGTLVTVSS

SEQ ID NO: 198 - protein, 118 aa, synthetic construct; identical to SEQ ID NO: 24
  REGION 1..118: note = Clone A63_Variable heavy chain

SEQ ID NO: 199 - protein, 118 aa, synthetic construct
  REGION 1..118: note = Clone A71_Variable heavy chain
EVQLVESGGGLVKPGGSLRLSCAASGFTFSSYAMNWVRQAPGKGLEWVSTITTGGSYTYYADSVHGRFTISRDNAKNSLYLQMNSLRAEDTAVYYCARQDGNFLMDYWGQGTLVTVSS

SEQ ID NO: 200 - protein, 118 aa, synthetic construct
  REGION 1..118: note = Clone A74_Variable heavy chain
EVQLVESGGGLVKPGGSLRLSCAASGFTFSSYAMHWVRQAPGKGLEWVSTITTGGSYTYYADSVQGRFTISRDNAKNSLYLQMNSLRAEDTAVYYCARQDGNFLMDYWGQGTLVTVSS

SEQ ID NO: 201 - protein, 16 aa, synthetic construct
  REGION 1..16: note = Clone A25_Variable light chain CDR 1
KSSQSLLDRDGKTYLN

SEQ ID NO: 202 - protein, 17 aa, synthetic construct
  REGION 1..17: note = Clone A71_Variable heavy chain CDR 2
TITTGGSYTYYADSVHG

SEQ ID NO: 203 - protein, 5 aa, synthetic construct
  REGION 1..5: note = Clone A74_Variable heavy chain CDR 1
SYAMH